European Patent Application EP 4 644 421 A1, published November 5, 2025. Title: 抗CD94的抗体及其应用. Applicant: 合肥天港免疫药物有限公司. The sequence listing filed with the application follows.

SEQUENCE LISTING (53 sequences)

SEQ ID NO: 1 - protein, 8 aa, synthetic construct
GFNIKDTY

SEQ ID NO: 2 - protein, 8 aa, synthetic construct
IDPANVNT

SEQ ID NO: 3 - protein, 11 aa, synthetic construct
VGGRGHTWFAY

SEQ ID NO: 4 - protein, 6 aa, synthetic construct
QDITNY

SEQ ID NO: 5 - protein, 9 aa, synthetic construct
QQGNTLPYT

SEQ ID NO: 6 - protein, 25 aa, synthetic construct
EVQLQQSGAELVMPGASVKLSCTAS

SEQ ID NO: 7 - protein, 17 aa, synthetic construct
MHWVMQRPEQGLEWIGR

SEQ ID NO: 8 - protein, 38 aa, synthetic construct
NYDPRFQGKATITADTSSNTAYLQFSSLTSEDTAVYYC

SEQ ID NO: 9 - protein, 11 aa, synthetic construct
WGQGTLVTVSA

SEQ ID NO: 10 - protein, 26 aa, synthetic construct
DIQMTQTTSSLSASLGDRVTISCRAS

SEQ ID NO: 11 - protein, 17 aa, synthetic construct
LNWYQQKPDGTVKLLIY

SEQ ID NO: 12 - protein, 36 aa, synthetic construct
RLHSGVPSRFSGSGSGTDYSLTISNLEQEDIATYFC

SEQ ID NO: 13 - protein, 10 aa, synthetic construct
FGGGTKLEIK

SEQ ID NO: 14 - protein, 25 aa, synthetic construct [sequence omitted]

SEQ ID NO: 15 - protein, 17 aa, synthetic construct
MHWVRQAPGQGLEWIGR

SEQ ID NO: 16 - protein, 38 aa, synthetic construct
NYDQKFQGRVTMTRDTSTSTVYMELSSLRSEDTAVYYC

SEQ ID NO: 17 - protein, 11 aa, synthetic construct
WGQGTTVTVSS

SEQ ID NO: 18 - protein, 26 aa, synthetic construct [sequence omitted]

SEQ ID NO: 19 - protein, 17 aa, synthetic construct
LNWYQQKPGKAPKLLIY

SEQ ID NO: 20 - protein, 36 aa, synthetic construct
RLHSGVPSRFSGSGSGTDYTLTISSLQPEDFATYYC

SEQ ID NO: 21 - protein, 10 aa, synthetic construct
FGQGTKLEIK

SEQ ID NO: 22 - protein, 118 aa, synthetic construct
EVQLQQSGAELVMPGASVKLSCTASGFNIKDTYMHWVMQRPEQGLEWIGRIDPANVNTNYDPRFQGKATITADTSSNTAYLQFSSLTSEDTAVYYCVGGRGHTWFAYWGQGTLVTVSA

SEQ ID NO: 23 - protein, 107 aa, synthetic construct
DIQMTQTTSSLSASLGDRVTISCRASQDITNYLNWYQQKPDGTVKLLIYYTSRLHSGVPSRFSGSGSGTDYSLTISNLEQEDIATYFCQQGNTLPYTFGGGTKLEIK

SEQ ID NO: 24 - protein, 118 aa, synthetic construct
QVQLVQSGAEVKKPGASVKVSCKASGFNIKDTYMHWVRQAPGQGLEWIGRIDPANVNTNYDQKFQGRVTMTRDTSTSTVYMELSSLRSEDTAVYYCVGGRGHTWFAYWGQGTTVTVSS

SEQ ID NO: 25 - protein, 107 aa, synthetic construct
DIQMTQSPSSLSASVGDRVTITCRASQDITNYLNWYQQKPGKAPKLLIYYTSRLHSGVPSRFSGSGSGTDYTLTISSLQPEDFATYYCQQGNTLPYTFGQGTKLEIK

SEQ ID NO: 26 - protein, 330 aa, synthetic construct
AKTTAPSVYPLAPVCGDTTGSSVTLGCLVKGYFPEPVTLTWNSGSLSSGVHTFPAVLQSDLYTLSSSVTVTSSTWPSQSITCNVAHPASSTKVDKKIEPRGPTIKPCPPCKCPAPNLLGGPSVFIFPPKIKDVLMISLSPIVTCVVVDVSEDDPDVQISWFVNNVEVHTAQTQTHREDYNSTLRVVSALPIQHQDWMSGKEFKCKVNNKDLPAPIERTISKPKGSVRAPQVYVLPPPEEEMTKKQVTLTCMVTDFMPEDIYVEWTNNGKTELNYKNTEPVLDSDGSYFMYSKLRVEKKNWVERNSYSCSVVHEGLHNHHTTKSFSRTPGK

SEQ ID NO: 27 - protein, 107 aa, synthetic construct
RADAAPTVSIFPPSSEQLTSGGASVVCFLNNFYPKDINVKWKIDGSERQNGVLNSWTDQDSKDSTYSMSSTLTLTKDEYERHNSYTCEATHKTSTSPIVKSFNRNEC

SEQ ID NO: 28 - protein, 330 aa, synthetic construct
ASTKGPSVFPLAPSSKSTSGGTAALGCLVKDYFPEPVTVSWNSGALTSGVHTFPAVLQSSGLYSLSSVVTVPSSSLGTQTYICNVNHKPSNTKVDKKVEPKSCDKTHTCPPCPAPELLGGPSVFLFPPKPKDTLMISRTPEVTCVVVAVSHEDPEVKFNWYVDGVEVHNAKTKPREEQYASTYRVVSVLTVLHQDWLNGKEYKCKVSNKALPAPIEKTISKAKGQPREPQVYTLPPSREEMTKNQVSLTCLVKGFYPSDIAVEWESNGQPENNYKTTPPVLDSDGSFFLYSKLTVDKSRWQQGNVFSCSVMHEALHNHYTQKSLSLSPGK

SEQ ID NO: 29 - protein, 107 aa, synthetic construct [sequence omitted]

SEQ ID NO: 30 - protein, 327 aa, synthetic construct
ASTKGPSVFPLAPCSRSTSESTAALGCLVKDYFPEPVTVSWNSGALTSGVHTFPAVLQSSGLYSLSSVVTVPSSSLGTKTYTCNVDHKPSNTKVDKRVESKYGPPCPPCPAPEFLGGPSVFLFPPKPKDTLMISRTPEVTCVVVDVSQEDPEVQFNWYVDGVEVHNAKTKPREEQFNSTYRVVSVLTVLHQDWLNGKEYKCKVSNKGLPSSIEKTISKAKGQPREPQVYTLPPSQEEMTKNQVSLTCLVKGFYPSDIAVEWESNGQPENNYKTTPPVLDSDGSFFLYSRLTVDKSRWQEGNVFSCSVMHEALHNHYTQKSLSLSLGK

SEQ ID NO: 31 - protein, 107 aa, synthetic construct [sequence omitted]

SEQ ID NO: 32 - protein, 448 aa, synthetic construct
EVQLQQSGAELVMPGASVKLSCTASGFNIKDTYMHWVMQRPEQGLEWIGRIDPANVNTNYDPRFQGKATITADTSSNTAYLQFSSLTSEDTAVYYCVGGRGHTWFAYWGQGTLVTVSAAKTTAPSVYPLAPVCGDTTGSSVTLGCLVKGYFPEPVTLTWNSGSLSSGVHTFPAVLQSDLYTLSSSVTVTSSTWPSQSITCNVAHPASSTKVDKKIEPRGPTIKPCPPCKCPAPNLLGGPSVFIFPPKIKDVLMISLSPIVTCVVVDVSEDDPDVQISWFVNNVEVHTAQTQTHREDYNSTLRVVSALPIQHQDWMSGKEFKCKVNNKDLPAPIERTISKPKGSVRAPQVYVLPPPEEEMTKKQVTLTCMVTDFMPEDIYVEWTNNGKTELNYKNTEPVLDSDGSYFMYSKLRVEKKNWVERNSYSCSVVHEGLHNHHTTKSFSRTPGK

SEQ ID NO: 33 - protein, 214 aa, synthetic construct
DIQMTQTTSSLSASLGDRVTISCRASQDITNYLNWYQQKPDGTVKLLIYYTSRLHSGVPSRFSGSGSGTDYSLTISNLEQEDIATYFCQQGNTLPYTFGGGTKLEIKRADAAPTVSIFPPSSEQLTSGGASVVCFLNNFYPKDINVKWKIDGSERQNGVLNSWTDQDSKDSTYSMSSTLTLTKDEYERHNSYTCEATHKTSTSPIVKSFNRNEC

SEQ ID NO: 34 - protein, 448 aa, synthetic construct
EVQLQQSGAELVMPGASVKLSCTASGFNIKDTYMHWVMQRPEQGLEWIGRIDPANVNTNYDPRFQGKATITADTSSNTAYLQFSSLTSEDTAVYYCVGGRGHTWFAYWGQGTLVTVSAASTKGPSVFPLAPSSKSTSGGTAALGCLVKDYFPEPVTVSWNSGALTSGVHTFPAVLQSSGLYSLSSVVTVPSSSLGTQTYICNVNHKPSNTKVDKKVEPKSCDKTHTCPPCPAPELLGGPSVFLFPPKPKDTLMISRTPEVTCVVVAVSHEDPEVKFNWYVDGVEVHNAKTKPREEQYASTYRVVSVLTVLHQDWLNGKEYKCKVSNKALPAPIEKTISKAKGQPREPQVYTLPPSREEMTKNQVSLTCLVKGFYPSDIAVEWESNGQPENNYKTTPPVLDSDGSFFLYSKLTVDKSRWQQGNVFSCSVMHEALHNHYTQKSLSLSPGK

SEQ ID NO: 35 - protein, 445 aa, synthetic construct
EVQLQQSGAELVMPGASVKLSCTASGFNIKDTYMHWVMQRPEQGLEWIGRIDPANVNTNYDPRFQGKATITADTSSNTAYLQFSSLTSEDTAVYYCVGGRGHTWFAYWGQGTLVTVSAASTKGPSVFPLAPCSRSTSESTAALGCLVKDYFPEPVTVSWNSGALTSGVHTFPAVLQSSGLYSLSSVVTVPSSSLGTKTYTCNVDHKPSNTKVDKRVESKYGPPCPPCPAPEFLGGPSVFLFPPKPKDTLMISRTPEVTCVVVDVSQEDPEVQFNWYVDGVEVHNAKTKPREEQFNSTYRVVSVLTVLHQDWLNGKEYKCKVSNKGLPSSIEKTISKAKGQPREPQVYTLPPSQEEMTKNQVSLTCLVKGFYPSDIAVEWESNGQPENNYKTTPPVLDSDGSFFLYSRLTVDKSRWQEGNVFSCSVMHEALHNHYTQKSLSLSLGK

SEQ ID NO: 36 - protein, 214 aa, synthetic construct
DIQMTQTTSSLSASLGDRVTISCRASQDITNYLNWYQQKPDGTVKLLIYYTSRLHSGVPSRFSGSGSGTDYSLTISNLEQEDIATYFCQQGNTLPYTFGGGTKLEIKRTVAAPSVFIFPPSDEQLKSGTASVVCLLNNFYPREAKVQWKVDNALQSGNSQESVTEQDSKDSTYSLSSTLTLSKADYEKHKVYACEVTHQGLSSPVTKSFNRGEC

SEQ ID NO: 37 - protein, 445 aa, synthetic construct
QVQLVQSGAEVKKPGASVKVSCKASGFNIKDTYMHWVRQAPGQGLEWIGRIDPANVNTNYDQKFQGRVTMTRDTSTSTVYMELSSLRSEDTAVYYCVGGRGHTWFAYWGQGTTVTVSSASTKGPSVFPLAPCSRSTSESTAALGCLVKDYFPEPVTVSWNSGALTSGVHTFPAVLQSSGLYSLSSVVTVPSSSLGTKTYTCNVDHKPSNTKVDKRVESKYGPPCPPCPAPEFLGGPSVFLFPPKPKDTLMISRTPEVTCVVVDVSQEDPEVQFNWYVDGVEVHNAKTKPREEQFNSTYRVVSVLTVLHQDWLNGKEYKCKVSNKGLPSSIEKTISKAKGQPREPQVYTLPPSQEEMTKNQVSLTCLVKGFYPSDIAVEWESNGQPENNYKTTPPVLDSDGSFFLYSRLTVDKSRWQEGNVFSCSVMHEALHNHYTQKSLSLSLGK

SEQ ID NO: 38 - protein, 214 aa, synthetic construct
DIQMTQSPSSLSASVGDRVTITCRASQDITNYLNWYQQKPGKAPKLLIYYTSRLHSGVPSRFSGSGSGTDYTLTISSLQPEDFATYYCQQGNTLPYTFGQGTKLEIKRTVAAPSVFIFPPSDEQLKSGTASVVCLLNNFYPREAKVQWKVDNALQSGNSQESVTEQDSKDSTYSLSSTLTLSKADYEKHKVYACEVTHQGLSSPVTKSFNRGEC

SEQ ID NO: 39 - protein, 179 aa, synthetic construct
MAVFKTTLWRLISGTLGIICLSLMATLGILLKNSFTKLSIEPAFTPGPNIELQKDSDCCSCQEKWVGYRCNCYFISSEQKTWNESRHLCASQKSSLLQLQNTDELDFMSSSQQFYWIGLSYSEEHTAWLWENGSALSQYLFPSFETFNTKNCIAYNPNGNALDESCEDKNRYICKQQLI

SEQ ID NO: 40 - DNA, 537 bp, synthetic construct
  source 1..537: mol_type = other DNA
atggcagtctttaagaccacactgtggaggctgataagcggcaccctggggatcatatgcctgtcacttatggctactctcggcatcttgctgaagaacagtttcaccaagctgagcatcgagccagctttcacccccggtcccaacatcgagctccagaaggattccgactgttgctcctgccaggaaaagtgggtgggctacaggtgtaactgctatttcatatcctcagagcagaagacatggaacgaatcccgacatctgtgcgccagccagaagtcaagcttgctgcagctccagaacaccgatgagcttgactttatgagctcctctcagcagttctattggattgggttgagctattctgaagagcatactgcatggttgtgggaaaacggctcagccctctcacaatatcttttcccttcatttgaaacctttaacaccaagaattgcattgcctataacccaaatggcaacgcactggatgagtcctgcgaagataaaaaccgatacatctgtaagcagcagcttatc

SEQ ID NO: 41 - protein, 233 aa, synthetic construct
MDNQGVIYSDLNLPPNPKRQQRKPKGNKNSILATEQEITYAELNLQKASQDFQGNDKTYHCKDLPSAPEKLIVGILGIICLILMASVVTIVVIPSTLIQRHNNSSLNTRTQKARHCGHCPEEWITYSNSCYYIGKERRTWEESLLACTSKNSSLLSIDNEEEMKFLSIISPSSWIGVFRNSSHHPWVTMNGLAFKHEIKDSDNAELNCAVLQVNRLKSAQCGSSIIYHCKHKL

SEQ ID NO: 42 - DNA, 699 bp, synthetic construct
  source 1..699: mol_type = other DNA
atggacaaccagggcgtgatctattctgacttgaacctgcctcccaacccaaaacgccagcagagaaagccaaaggggaataagaacagtatcctcgccacagagcaggagattacttacgccgagctcaacctgcagaaggcatctcaggattttcaaggaaacgataaaacctaccactgcaaagacttgccttccgctcctgaaaagctgatcgtcggcattctcggtatcatctgcctcatccttatggcctccgtggtgacaattgtcgtcattccatccacactgatccaacgacacaataattcttctctgaataccaggacacagaaggccagacattgcggccattgtcctgaggaatggatcacctattccaactcttgttattatattgggaaggagcgcagaacttgggaagaatctctgctcgcttgcacatctaagaacagttctctcctgtccatcgacaatgaagaagagatgaagtttctgagcatcatttctccctcctcctggatcggggtgtttcgtaactcaagtcatcatccttgggtgactatgaatggattggcctttaagcacgaaatcaaggattccgataatgctgagcttaactgtgccgtcctgcaagtcaataggctgaagtccgctcagtgcggctcctctattatataccactgcaaacataagctg

SEQ ID NO: 43 - protein, 454 aa, synthetic construct
QVQLVQSGAEVKKPGASVKVSCKASGYTFTSYWMNWVRQAPGQGLEWMGRIDPYDSETHYAQKLQGRVTMTTDTSTSTAYMELRSLRSDDTAVYYCARGGYDFDVGTLYWFFDVWGQGTTVTVSASTKGPSVFPLAPSSKSTSGGTAALGCLVKDYFPEPVTVSWNSGALTSGVHTFPAVLQSSGLYSLSSVVTVPSSSLGTQTYICNVNHKPSNTKVDKKVEPKSCDKTHTCPPCPAPELLGGPSVFLFPPKPKDTLMISRTPEVTCVVVAVSHEDPEVKFNWYVDGVEVHNAKTKPREEQYASTYRVVSVLTVLHQDWLNGKEYKCKVSNKALPAPIEKTISKAKGQPREPQVYTLPPSREEMTKNQVSLTCLVKGFYPSDIAVEWESNGQPENNYKTTPPVLDSDGSFFLYSKLTVDKSRWQQGNVFSCSVMHEALHNHYTQKSLSLSPGK

SEQ ID NO: 44 - protein, 214 aa, synthetic construct
DIQMTQSPSSLSASVGDRVTITCRASENIYSYLAWYQQKPGKAPKLLIYNAKTLAEGVPSRFSGSGSGTDFTLTISSLQPEDFATYYCQHHYGTPRTFGGGTKVEIKRTVAAPSVFIFPPSDEQLKSGTASVVCLLNNFYPREAKVQWKVDNALQSGNSQESVTEQDSKDSTYSLSSTLTLSKADYEKHKVYACEVTHQGLSSPVTKSFNRGEC

SEQ ID NO: 45 - protein, 446 aa, synthetic construct
EVQLVESGGGLVKPGGSLRLSCAASGFTFSSYAMSWVRQAPGKGLEWVSEISSGGSYTYYADSVKGRFTISRDNAKNSLYLQMNSLRAEDTAVYYCARHGDYPRFFDVWGQGTTVTVSSASTKGPSVFPLAPCSRSTSESTAALGCLVKDYFPEPVTVSWNSGALTSGVHTFPAVLQSSGLYSLSSVVTVPSSSLGTKTYTCNVDHKPSNTKVDKRVESKYGPPCPPCPAPEFLGGPSVFLFPPKPKDTLMISRTPEVTCVVVDVSQEDPEVQFNWYVDGVEVHNAKTKPREEQFNSTYRVVSVLTVLHQDWLNGKEYKCKVSNKGLPSSIEKTISKAKGQPREPQVYTLPPSQEEMTKNQVSLTCLVKGFYPSDIAVEWESNGQPENNYKTTPPVLDSDGSFFLYSRLTVDKSRWQEGNVFSCSVMHEALHNHYTQKSLSLSLGK

SEQ ID NO: 46 - protein, 214 aa, synthetic construct
EIVLTQSPATLSLSPGERATLSCSASSSVSSYIYWYQQKPGQAPRLLIYLTSNLASGIPARFSGSGSGTDFTLTISSLEPEDFAVYYCQQWSGNPYTFGQGTKLEIKRTVAAPSVFIFPPSDEQLKSGTASVVCLLNNFYPREAKVQWKVDNALQSGNSQESVTEQDSKDSTYSLSSTLTLSKADYEKHKVYACEVTHQGLSSPVTKSFNRGEC

SEQ ID NO: 47 - protein, 451 aa, synthetic construct
QVQLVQSGAEVKKPGASVKVSCKASGYTFTSYWMNWVRQAPGQGLEWMGRIDPYDSETHYAQKLQGRVTMTTDTSTSTAYMELRSLRSDDTAVYYCARGGYDFDVGTLYWFFDVWGQGTTVTVSASTKGPSVFPLAPCSRSTSESTAALGCLVKDYFPEPVTVSWNSGALTSGVHTFPAVLQSSGLYSLSSVVTVPSSSLGTKTYTCNVDHKPSNTKVDKRVESKYGPPCPPCPAPEFLGGPSVFLFPPKPKDTLMISRTPEVTCVVVDVSQEDPEVQFNWYVDGVEVHNAKTKPREEQFNSTYRVVSVLTVLHQDWLNGKEYKCKVSNKGLPSSIEKTISKAKGQPREPQVYTLPPSQEEMTKNQVSLTCLVKGFYPSDIAVEWESNGQPENNYKTTPPVLDSDGSFFLYSRLTVDKSRWQEGNVFSCSVMHEALHNHYTQKSLSLSLGK

SEQ ID NO: 48 - protein, 214 aa, synthetic construct; identical to SEQ ID NO: 44

SEQ ID NO: 49 - protein, 379 aa, synthetic construct
PKSCDKTHTCPPCPAPELLGGPSVFLFPPKPKDTLMISRTPEVTCVVVAVSHEDPEVKFNWYVDGVEVHNAKTKPREEQYASTYRVVSVLTVLHQDWLNGKEYKCKVSNKALPAPIEKTISKAKGQPREPQVYTLPPSREEMTKNQVSLWCLVKGFYPSDIAVEWESNGQPENNYKTTPPVLDSDGSFFLYSKLTVDKSRWQQGNVFSCSVMHEALHNHYTQKSLSLSPGKKNSFTKLSIEPAFTPGPNIELQKDSDCCSCQEKWVGYRCNCYFISSEQKTWNESRHLCASQKSSLLQLQNTDELDFMSSSAQFYWIGLSYSEEHTAWLWENGSALSQYLFPSFETFNTKNCIAYNPNGNALDESCEDKNRYICKQQLI

SEQ ID NO: 50 - protein, 371 aa, synthetic construct
PKSCDKTHTCPPCPAPELLGGPSVFLFPPKPKDTLMISRTPEVTCVVVAVSHEDPEVKFNWYVDGVEVHNAKTKPREEQYASTYRVVSVLTVLHQDWLNGKEYKCKVSNKALPAPIEKTISKAKGQPREPQVYTLPPSREEMTKNQVSLSCAVKGFYPSDIAVEWESNGQPENNYKTTPPVLDSDGSFFLVSKLTVDKSRWQQGNVFSCSVMHEALHNHYTQKSLSLSPGKPSTLIQRHNNSSLNTRTQKARHCGHCPEEWITYSNSCYYIGKERRTWEESLLACTSKNSSLLSIDNEEEMKFLSIISPSSWIGVFRNSSHHPWVTMNGLAFKHEIKDSDNAELNCAVLQVNRLKSAQCGSSIIYHCKHKL

SEQ ID NO: 51 - protein, 358 aa, synthetic construct
MVDGTLLLLLSEALALTQTWAGSHSLKYFHTSVSRPGRGEPRFISVGYVDDTQFVRFDNDAASPRMVPRAPWMEQEGSEYWDRETRSARDTAQIFRVNLRTLRGYYNQSEAGSHTLQWMHGCELGPDGRFLRGYEQFAYDGKDYLTLNEDLRSWTAVDTAAQISEQKSNDASEAEHQRAYLEDTCVEWLHKYLEKGKETLLHLEPPKTHVTHHPISDHEATLRCWALGFYPAEITLTWQQDGEGHTQDTELVETRPAGDGTFQKWAAVVVPSGEEQRYTCHVQHEGLPEPVTLRWKPASQPTIPIVGIIAGLVLLGSVVSGAVVAAVIWRKKSSGGKGGSYSKAEWSDSAQGSESHSL

SEQ ID NO: 52 - DNA, 1074 bp, synthetic construct
  source 1..1074: mol_type = other DNA
atggtggatggaacactgctcctgttgctttctgaggctctggctttgactcagacttgggccgggagccatagcctgaaatatttccacacaagtgtttctaggcctggaagaggcgaaccaaggttcatcagtgtcggctatgtggacgacactcagttcgtgcgattcgataacgacgctgcaagtcctcgcatggtaccccgtgctccatggatggagcaggaaggaagtgaatattgggaccgcgaaacacggagcgcacgcgataccgcccagattttcagggtgaacctccgtaccctgaggggctactataatcagagcgaggccggctcccatactttgcagtggatgcacgggtgcgagctgggacccgatggccgttttctgcggggttacgagcagttcgcctacgacggcaaggactatctgacactgaacgaagatctcaggagctggacagctgtcgacaccgctgcccagataagtgagcagaaaagcaatgacgcttcagaggctgagcatcagagggcatacttggaggatacctgcgtggagtggttgcataagtatctcgagaagggcaaagagaccttgctgcatttggagccccccaaaacacatgtgacccaccaccccattagtgatcatgaagccaccctccgatgctgggccctcggattctatccagccgagattactctgacatggcaacaggatggagagggtcatacccaggacaccgagctggtcgagacccgtcccgctggggacggtacattccagaagtgggccgcagtggtggtccctagcggcgaagagcagcgatacacatgtcatgtgcagcatgaaggtctgcctgaacctgttaccctgcggtggaaacctgcatctcagcccactatccctattgtgggcatcatcgctggcctcgtattgttgggaagcgtggtgtcaggcgctgtggtggctgctgtgatctggcggaagaaaagctccggaggcaagggcgggtcatattctaaggcagaatggtccgatagcgctcagggtagtgagtctcactctctg

SEQ ID NO: 53 - protein, 380 aa, synthetic construct
NSFTKLSIEPAFTPGPNIELQKDSDCCSCQEKWVGYRCNCYFISSEQKTWNESRHLCASQKSSLLQLQNTDELDFMSSSQQFYWIGLSYSEEHTAWLWENGSALSQYLFPSFETFNTKNCIAYNPNGNALDESCEDKNRYICKQQLILEPKSCDKTHTCPPCPAPELLGGPSVFLFPPKPKDTLMISRTPEVTCVVVDVSHEDPEVKFNWYVDGVEVHNAKTKPREEQYNSTYRVVSVLTVLHQDWLNGKEYKCKVSNKALPAPIEKTISKAKGQPREPQVYTLPPSRDELTKNQVSLTCLVKGFYPSDIAVEWESNGQPENNYKTTPPVLDSDGSFFLYSKLTVDKSRWQQGNVFSCSVMHEALHNHYTQKSLSLSPGK